European Patent Specification EP 3 887 533 B1, published January 4, 2023. Title: Method for the fermentative production of L-lysine. Applicant: Evonik Operations GmbH. The sequence listing filed with the application follows.

SEQUENCE LISTING (19 sequences)

SEQ ID NO: 1 - DNA, 2351 bp, Corynebacterium glutamicum ATCC13032
  CDS (1001)..(1348): coding sequence of NCgl0275 (whiB4)
  misc_feature (1349)..(1351): taa stop codon
agccctgcaaatccacaccatcatgctcatagaacctgcgatcctcaatcgaaacgatcgcatccttcatcgacgtagaaatctgatcacccccaacctcaaaccgccgctgcgcataaatataagcaatcggctggtcagtggaatcagtaatcgtcgtgacgcccggcccgcgaccatccgtcagatctgaaaggttggtctgcatcgtgtcattggtacgcgcaaccgcaacgccagaaagactagcgaaaggcacaagtgcgagcgcaccaaggacgccagcggcgactgtagatgcaacgagctttgtcagagaattcgtggtggacactccaacagcctagcgataaccccgggaatcgtgaacccaagactccaacaatgtcagccaatctttatttattcgactgtgcgttactgctgacagtcggcatgctttgggaatccaccaggcaagctataggggactgtagagctgacgttcggaaaacgtgcagaaaaccacgaactgcagtccggaaagcgccccactggcccttcgccggcagccacagaggggttagaccatttattcgcaactgtgcttacacccaagaattctccaacaagaaaaatccctctatcaacattttaagtgaatgaccttaagggtttgcggaatgcgatccatgttccaactcgcctcaagcggtatgtgtgaagcaggtttgaagccagtgatgacctctgatggggttagtttgtggcaatttcggggctggctgaaatgcctaattttccaaaactgaatttaatgagttgagctgtggtaagactagtgaactgcagatatgttggacaattgtaaagtcctctcgttggaggcttggcagtgtggccataaaagtattgcccccgttggtgtgatgcattcgacagcaaattggctgtgtgactacacttgcgagtgtattaagtattaggccgtgcatatgtagcgcattttaaggagattgtcatgacgtctgtgattccagagcagcgcaacaaccccttttatagggacagcgccacaattgcttcctcggaccacacagagcgtggtgagtgggtcactcaggcaaagtgtcgaaatggcgacccagatgcattgtttgttcgtggtgcagcgcaacgccgagcagcagcaatttgccgccactgccctgtagccatgcagtgctgcgccgatgccttagataacaaggtggaattcggagtctggggaggcctgaccgagcgccagcgccgtgcattgcttcgaaagaagccgcacattactaactgggctgaatatttggctcaggggggcgagatcgccggggtttaattaatttcaagggctggccattaacgtggtcggcttttttgattcagggcgcaccccaggcgcaccccaggcgcaccccagcgcaccacaggcgcaccccagcgcaccacaggcgcaccagcccagcacaagagccaacgcaagtgtcaggcacgccagcaaaggggctagcaagaagcacgcccccgaagccttagaaatgcgttccccggtaggatgattgccatgactaaatgggaatacgcaactgtgcctttgattacgcatgcaactaagcagatcctcgatacttggggtgaggacggctgggagttggtctcggtcatgcctggtatgaaccctgagaacctcgttgcttacatgaagcgtgaggtggcttagttcttatggcttctaattccgaacgccttgcagagctgggcatttctcttccttccgttgcagcgcctgttgctgcgtatgttcctgcgattcagaccggtaaccaggtgtggacttctggtcagctgcctttcgttgatggtcagcttccggccaccggcaaggttggcgctgaggtttccgctgaggatgcggagaagttggctcgtgcggctgcgctaaacgctcttgctgcgattgatgcgcttgttggcattgataaggtcactcgcgttttgaagattgttggtttcgtggcgtctgctgatgatttcagtggtcagcctgctgtcgtcaacggtgcttccaatttgatgggtgaggttttcggcgaggctggggcgcatgcgcgttctgctgtgggcgtggcggagttgccgctcaactcgcctgtcgaggtcgaggttatcgtcgagatcgcgcagtagcacgcttttcgacgcaaaatgccggttccgcacttcgtgcgaaaccggcatttttaaattgaccctatcgtccccttagtgttcgtaagtagaaagatcgtggtcttttgattctctggtgattgcgatggcgatgatggacactagggaca

SEQ ID NO: 2 - protein, 116 aa, Corynebacterium glutamicum ATCC13032
MTSVIPEQRNNPFYRDSATIASSDHTERGEWVTQAKCRNGDPDALFVRGAAQRRAAAICRHCPVAMQCCADALDNKVEFGVWGGLTERQRRALLRKKPHITNWAEYLAQGGEIAGV

SEQ ID NO: 3 - DNA, 1266 bp, Corynebacterium glutamicum ATCC13032
  CDS (1)..(1263): cds of aspartokinase gene
  misc_feature (1264)..(1266): taa stop codon
gtggccctggtcgtacagaaatatggcggttcctcgcttgagagtgcggaacgcattagaaacgtcgctgaacggatcgttgccaccaagaaggctggaaatgatgtcgtggttgtctgctccgcaatgggagacaccacggatgaacttctagaacttgcagcggcagtgaatcccgttccgccagctcgtgaaatggatatgctcctgactgctggtgagcgtatttctaacgctctcgtcgccatggctattgagtcccttggcgcagaagcccaatctttcacgggctctcaggctggtgtgctcaccaccgagcgccacggaaacgcacgcattgttgatgtcactccaggtcgtgtgcgtgaagcactcgatgagggcaagatctgcattgttgctggtttccagggtgttaataaagaaacccgcgatgtcaccacgttgggtcgtggtggttctgacaccactgcagttgcgttggcagctgctttgaacgctgatgtgtgtgagatttactcggacgttgacggtgtgtataccgctgacccgcgcatcgttcctaatgcacagaagctggaaaagctcagcttcgaagaaatgctggaacttgctgctgttggctccaagattttggtgctgcgcagtgttgaatacgctcgtgcattcaatgtgccacttcgcgtacgctcgtcttatagtaatgatcccggcactttgattgccggctctatggaggatattcctgtggaagaagcagtccttaccggtgtcgcaaccgacaagtccgaagccaaagtaaccgttctgggtatttccgataagccaggcgaggctgcgaaggttttccgtgcgttggctgatgcagaaatcaacattgacatggttctgcagaacgtctcttctgtagaagacggcaccaccgacatcaccttcacctgccctcgttccgacggccgccgcgcgatggagatcttgaagaagcttcaggttcagggcaactggaccaatgtgctttacgacgaccaggtcggcaaagtctccctcgtgggtgctggcatgaagtctcacccaggtgttaccgcagagttcatggaagctctgcgcgatgtcaacgtgaacatcgaattgatttccacctctgagattcgtatttccgtgctgatccgtgaagatgatctggatgctgctgcacgtgcattgcatgagcagttccagctgggcggcgaagacgaagccgtcgtttatgcaggcaccggacgctaa

SEQ ID NO: 4 - protein, 421 aa, Corynebacterium glutamicum ATCC13032
MALVVQKYGGSSLESAERIRNVAERIVATKKAGNDVVVVCSAMGDTTDELLELAAAVNPVPPAREMDMLLTAGERISNALVAMAIESLGAEAQSFTGSQAGVLTTERHGNARIVDVTPGRVREALDEGKICIVAGFQGVNKETRDVTTLGRGGSDTTAVALAAALNADVCEIYSDVDGVYTADPRIVPNAQKLEKLSFEEMLELAAVGSKILVLRSVEYARAFNVPLRVRSSYSNDPGTLIAGSMEDIPVEEAVLTGVATDKSEAKVTVLGISDKPGEAAKVFRALADAEINIDMVLQNVSSVEDGTTDITFTCPRSDGRRAMEILKKLQVQGNWTNVLYDDQVGKVSLVGAGMKSHPGVTAEFMEALRDVNVNIELISTSEIRISVLIREDDLDAAARALHEQFQLGGEDEAVVYAGTGR

SEQ ID NO: 5 - DNA, 1631 bp, artificial sequence
  nucleotide sequence comprising a deletion of the cds of the whiB4 gene of Corynebacterium glutamicum ATCC13032 and the adjoining stop codon
  misc_feature (1)..(16): sequence required for Gibson assembly
  misc_feature (17)..(816): sequence upstream of the site of deletion (5'-flanking sequence)
  misc_feature (811)..(822): sequence attgtcttaatt
  misc_feature (816)..(817): positions identifying the site of deletion of the coding sequence and the adjoining stop codon of the whiB4 gene
  misc_feature (817)..(1616): sequence downstream of the site of deletion (3'-flanking sequence)
  misc_feature (1617)..(1631): sequence required for Gibson assembly
ggtacccggggatcctgtctgcatcgtgtcattggtacgcgcaaccgcaacgccagaaagactagcgaaaggcacaagtgcgagcgcaccaaggacgccagcggcgactgtagatgcaacgagctttgtcagagaattcgtggtggacactccaacagcctagcgataaccccgggaatcgtgaacccaagactccaacaatgtcagccaatctttatttattcgactgtgcgttactgctgacagtcggcatgctttgggaatccaccaggcaagctataggggactgtagagctgacgttcggaaaacgtgcagaaaaccacgaactgcagtccggaaagcgccccactggcccttcgccggcagccacagaggggttagaccatttattcgcaactgtgcttacacccaagaattctccaacaagaaaaatccctctatcaacattttaagtgaatgaccttaagggtttgcggaatgcgatccatgttccaactcgcctcaagcggtatgtgtgaagcaggtttgaagccagtgatgacctctgatggggttagtttgtggcaatttcggggctggctgaaatgcctaattttccaaaactgaatttaatgagttgagctgtggtaagactagtgaactgcagatatgttggacaattgtaaagtcctctcgttggaggcttggcagtgtggccataaaagtattgcccccgttggtgtgatgcattcgacagcaaattggctgtgtgactacacttgcgagtgtattaagtattaggccgtgcatatgtagcgcattttaaggagattgtcttaatttcaagggctggccattaacgtggtcggcttttttgattcagggcgcaccccaggcgcaccccaggcgcaccccagcgcaccacaggcgcaccccagcgcaccacaggcgcaccagcccagcacaagagccaacgcaagtgtcaggcacgccagcaaaggggctagcaagaagcacgcccccgaagccttagaaatgcgttccccggtaggatgattgccatgactaaatgggaatacgcaactgtgcctttgattacgcatgcaactaagcagatcctcgatacttggggtgaggacggctgggagttggtctcggtcatgcctggtatgaaccctgagaacctcgttgcttacatgaagcgtgaggtggcttagttcttatggcttctaattccgaacgccttgcagagctgggcatttctcttccttccgttgcagcgcctgttgctgcgtatgttcctgcgattcagaccggtaaccaggtgtggacttctggtcagctgcctttcgttgatggtcagcttccggccaccggcaaggttggcgctgaggtttccgctgaggatgcggagaagttggctcgtgcggctgcgctaaacgctcttgctgcgattgatgcgcttgttggcattgataaggtcactcgcgttttgaagattgttggtttcgtggcgtctgctgatgatttcagtggtcagcctgctgtcgtcaacggtgcttccaatttgatgggtgaggttttcggcgaggctggggcgcatgcgcgttctgctgtgggcgtggcggagttgccgagtcgacctgcaggc

SEQ ID NO: 6 - DNA, 1600 bp, artificial sequence
  nucleotide sequence comprising a deletion of part of the cds of the whiB4 gene of Corynebacterium glutamicum ATCC13032
  misc_feature (1)..(800): sequence upstream of the site of deletion (5'-flanking sequence)
  CDS (774)..(800): residual 5'-coding sequence
  misc_feature (794)..(807): sequence gcagcgcgccgggg
  misc_feature (800)..(801): positions identfying the site of deletion within the coding sequence of the whiB4 gene
  CDS (801)..(809): residual 3'-coding sequence
  misc_feature (801)..(1600): sequence downstream of the site of mutation (3'-flanking sequence)
  misc_feature (810)..(812): taa stop codon
accgcaacgccagaaagactagcgaaaggcacaagtgcgagcgcaccaaggacgccagcggcgactgtagatgcaacgagctttgtcagagaattcgtggtggacactccaacagcctagcgataaccccgggaatcgtgaacccaagactccaacaatgtcagccaatctttatttattcgactgtgcgttactgctgacagtcggcatgctttgggaatccaccaggcaagctataggggactgtagagctgacgttcggaaaacgtgcagaaaaccacgaactgcagtccggaaagcgccccactggcccttcgccggcagccacagaggggttagaccatttattcgcaactgtgcttacacccaagaattctccaacaagaaaaatccctctatcaacattttaagtgaatgaccttaagggtttgcggaatgcgatccatgttccaactcgcctcaagcggtatgtgtgaagcaggtttgaagccagtgatgacctctgatggggttagtttgtggcaatttcggggctggctgaaatgcctaattttccaaaactgaatttaatgagttgagctgtggtaagactagtgaactgcagatatgttggacaattgtaaagtcctctcgttggaggcttggcagtgtggccataaaagtattgcccccgttggtgtgatgcattcgacagcaaattggctgtgtgactacacttgcgagtgtattaagtattaggccgtgcatatgtagcgcattttaaggagattgtcatgacgtctgtgattccagagcagcgcgccggggtttaattaatttcaagggctggccattaacgtggtcggcttttttgattcagggcgcaccccaggcgcaccccaggcgcaccccagcgcaccacaggcgcaccccagcgcaccacaggcgcaccagcccagcacaagagccaacgcaagtgtcaggcacgccagcaaaggggctagcaagaagcacgcccccgaagccttagaaatgcgttccccggtaggatgattgccatgactaaatgggaatacgcaactgtgcctttgattacgcatgcaactaagcagatcctcgatacttggggtgaggacggctgggagttggtctcggtcatgcctggtatgaaccctgagaacctcgttgcttacatgaagcgtgaggtggcttagttcttatggcttctaattccgaacgccttgcagagctgggcatttctcttccttccgttgcagcgcctgttgctgcgtatgttcctgcgattcagaccggtaaccaggtgtggacttctggtcagctgcctttcgttgatggtcagcttccggccaccggcaaggttggcgctgaggtttccgctgaggatgcggagaagttggctcgtgcggctgcgctaaacgctcttgctgcgattgatgcgcttgttggcattgataaggtcactcgcgttttgaagattgttggtttcgtggcgtctgctgatgatttcagtggtcagcctgctgtcgtcaacggtgcttccaatttgatgggtgaggttttcggcgaggctggggcgcatgcgcgttctgctgtgggcgtg

SEQ ID NO: 7 - protein, 9 aa, artificial sequence
  Synthetic Construct
MTSVIPEQR

SEQ ID NO: 8 - DNA, 35 bp, artificial sequence
  primer
  misc_feature (1)..(35): primer 1f-NCgl0275
ggtacccggggatcctgtctgcatcgtgtcattgg

SEQ ID NO: 9 - DNA, 37 bp, artificial sequence
  primer
  misc_feature (1)..(37): primer 1r-NCgl0275
cccttgaaattaagacaatctccttaaaatgcgctac

SEQ ID NO: 10 - DNA, 35 bp, artificial sequence
  primer
  misc_feature (1)..(35): primer 2f-NCgl0275
taaggagattgtcttaatttcaagggctggccatt

SEQ ID NO: 11 - DNA, 33 bp, artificial sequence
  primer
  misc_feature (1)..(33): primer 2f-NCgl0275_2
gcctgcaggtcgactcggcaactccgccacgcc

SEQ ID NO: 12 - DNA, 829 bp, artificial sequence
  amplificate whiB4_up
ggtacccggggatcctgtctgcatcgtgtcattggtacgcgcaaccgcaacgccagaaagactagcgaaaggcacaagtgcgagcgcaccaaggacgccagcggcgactgtagatgcaacgagctttgtcagagaattcgtggtggacactccaacagcctagcgataaccccgggaatcgtgaacccaagactccaacaatgtcagccaatctttatttattcgactgtgcgttactgctgacagtcggcatgctttgggaatccaccaggcaagctataggggactgtagagctgacgttcggaaaacgtgcagaaaaccacgaactgcagtccggaaagcgccccactggcccttcgccggcagccacagaggggttagaccatttattcgcaactgtgcttacacccaagaattctccaacaagaaaaatccctctatcaacattttaagtgaatgaccttaagggtttgcggaatgcgatccatgttccaactcgcctcaagcggtatgtgtgaagcaggtttgaagccagtgatgacctctgatggggttagtttgtggcaatttcggggctggctgaaatgcctaattttccaaaactgaatttaatgagttgagctgtggtaagactagtgaactgcagatatgttggacaattgtaaagtcctctcgttggaggcttggcagtgtggccataaaagtattgcccccgttggtgtgatgcattcgacagcaaattggctgtgtgactacacttgcgagtgtattaagtattaggccgtgcatatgtagcgcattttaaggagattgtcttaatttcaaggg

SEQ ID NO: 13 - DNA, 828 bp, artificial sequence
  amplificate whiB4_down
taaggagattgtcttaatttcaagggctggccattaacgtggtcggcttttttgattcagggcgcaccccaggcgcaccccaggcgcaccccagcgcaccacaggcgcaccccagcgcaccacaggcgcaccagcccagcacaagagccaacgcaagtgtcaggcacgccagcaaaggggctagcaagaagcacgcccccgaagccttagaaatgcgttccccggtaggatgattgccatgactaaatgggaatacgcaactgtgcctttgattacgcatgcaactaagcagatcctcgatacttggggtgaggacggctgggagttggtctcggtcatgcctggtatgaaccctgagaacctcgttgcttacatgaagcgtgaggtggcttagttcttatggcttctaattccgaacgccttgcagagctgggcatttctcttccttccgttgcagcgcctgttgctgcgtatgttcctgcgattcagaccggtaaccaggtgtggacttctggtcagctgcctttcgttgatggtcagcttccggccaccggcaaggttggcgctgaggtttccgctgaggatgcggagaagttggctcgtgcggctgcgctaaacgctcttgctgcgattgatgcgcttgttggcattgataaggtcactcgcgttttgaagattgttggtttcgtggcgtctgctgatgatttcagtggtcagcctgctgtcgtcaacggtgcttccaatttgatgggtgaggttttcggcgaggctggggcgcatgcgcgttctgctgtgggcgtggcggagttgccgagtcgacctgcaggc

SEQ ID NO: 14 - DNA, 20 bp, artificial sequence
  primer
  misc_feature (1)..(20): primer DNCgl0275_seq_1
gccagtgatgacctctgatg

SEQ ID NO: 15 - DNA, 20 bp, artificial sequence
  primer
  misc_feature (1)..(20): primer DNCgl0275_seq_2
ttccgaacgccttgcagagc

SEQ ID NO: 16 - DNA, 20 bp, artificial sequence
  primer
  misc_feature (1)..(20): primer pCV22_1.p
aggtttcccgactggaaagc

SEQ ID NO: 17 - DNA, 20 bp, artificial sequence
  primer
  misc_feature (1)..(20): primer Ncgl0275_rev
gtggcggcaaattgctgctg

SEQ ID NO: 18 - DNA, 20 bp, artificial sequence
  primer
  misc_feature (1)..(20): primer NCgl0276_rev2
ataccaggcatgaccgagac

SEQ ID NO: 19 - DNA, 20 bp, artificial sequence
  primer
  misc_feature (1)..(20): primer Ncgl0274_fw
tgcaacgagctttgtcagag